European Patent Specification EP 3 665 186 B1, published October 4, 2023. Title: VP-60 RECOMBINANT PROTEIN AND RELATIVE METHOD OF PRODUCTION AND PURIFICATION. Applicant: ISTITUTO ZOOPROFILATTICO SPERIMENTALE UMBRIA E MARCHE. The sequence listing filed with the application follows.

SEQUENCE LISTING (6 sequences)

SEQ ID NO: 1 - protein, 588 aa, Baculoviridae
  R-VP60-His7
MEGKARTAPQSDAAGTATTASYPGTTTDGMDPGVVATTSVVTTENSSASIATAGIGGPPQQVDQQETWRTNFYYNDVFTWSVADAPGSILYTVQHSPQNNPFTAVLSQMYAGWAGGMQFRFIVAGSGVFGGRLVAAVIPPGIEIGPGLEVRQFPHVVIDARSLEPVTITMPDLRPNMYHPTGDPGLVPTLVLSVYNNLINPFGGSTSAIQVTVETRPSEDFEFVMIRAPSSKTVDSISPAGLLTTPVLTGVGNDNRWNGQIVGLQPVPGGFSTCNRHWNLNGSTYGWSSPRFADIDHRSGSASYPGNNATNVLQFWYANAGSAIDNPISQVAPDGFPDMSFVPFNGPGIPAAGWVGFGAIWNSNSGAPNVTTVQAYELGFATGAPGNLQPTTNTSGAQTVAKSIYAVVTGTGQSPAGLFVMASGIISTPNANAITYTPQPDRIVTTPGTPAAAPVGKNTPIMFASVVRRTGDVNATAGSTNGTQYGTGSQPLPVTIGLSLNNYSSALMPGQFFVWQLTFASGFMEIGLSVDGYFYAGTGASTTLIDLTELIDVRPVGPRPSKSTLVFNLGGAANGFSYVGGHHHHHHH

SEQ ID NO: 2 - DNA, 1767 bp, Baculoviridae
  RHDV-VP60-His7/pOET2C
atggagggcaaagcccgcacagcgccgcaaagcgatgcagcgggcactgctaccacagcatcagtccctggaaccacaaccgacggtatggatcctggcgtcgtggccacaaccagcgtggtcaccaccgagaattcatccgcgtcgattgcaacggcagggattggcggaccaccccaacaggtggaccaacaagagacatggagaacaaatttttattacaatgatgttttcacttggtcagtcgcagacgcccccggcagtatactttataccgtccagcattctccacaaaacaacccatttacagccgtactgagccagatgtacgctggctgggctggtggcatgcagtttcgcttcatagttgctggttcaggtgtgttcggtgggcgactggttgcagctgtgataccaccaggcattgagattggaccagggttggaggtcaggcaatttcctcatgttgtcatcgacgcccgttcacttgaacctgttaccatcaccatgccagacttgcgtcccaacatgtaccatccaactggtgaccctggtcttgtccccacactggtccttagtgtttacaacaatctcatcaacccgtttggagggtccaccagcgcaatccaggtgacggtggaaacaaggccgagtgaagactttgagttcgtgatgattcgagccccttctagcaagactgttgactcaatttcacctgcaggcctcctcacaaccccagttctcaccggggtcggtaatgacaacaggtggaacggccaaatagtgggactgcaaccggtgcccggagggttttctacatgcaacaggcattggaacttgaatggcagcacgtatggctggtcaagccctcggtttgctgacattgaccatcgaagtggcagtgcaagttaccctgggaacaacgcaaccaacgtgcttcagttttggtatgccaacgctggatctgcaattgacaaccccatctcccaggttgcaccggacggctttcctgacatgtcgttcgtgccctttaatggtcctggcatcccagccgcggggtgggtcggatttggtgcaatctggaacagcaacagcggtgctcccaacgttacgactgtgcaggcctatgagttaggttttgccactggggcaccaggcaacctccagcccactaccaacacttcaggtgcgcaaactgtcgccaaatccatttacgccgtggtaaccggtacaggccaaagcccagccgggttgtttgtgatggcctcgggcatcatctctaccccaaatgccaatgccatcacatacacacctcaaccagacagaattgtaaccacacccggcacaccagccgctgcacctgtgggtaaaaacacacccatcatgtttgcgtctgtcgttaggcgcaccggtgacgttaacgccacagctggatcaactaacggcactcagtatggcacaggctcccaaccactgccagtgacaattgggctttcgctcaacaactactcgtcagcactcatgcccggacagttcttcgtgtggcagttaacctttgcatctggtttcatggagattggtttaagtgtggacgggtatttttatgcaggaacaggggcctcaaccacactcattgacttgactgaactcattgatgttcgccctgtgggacccaggccatccaaaagcacactcgtgttcaacctggggggcgcagctaatggcttttcttatgtcggaggtcaccatcatcaccaccatcactag

SEQ ID NO: 3 - DNA, 35 bp, Baculoviridae
  RHDV/EcoRI-F
tgtgaattctataaataatggagggcaaagcccgc

SEQ ID NO: 4 - DNA, 26 bp, Baculoviridae
  RHDV/HindIII-R
caaaagcttcagacataagaaaagcc

SEQ ID NO: 5 - DNA, 22 bp, Baculoviridae
  RHDV/Pst-F
gttgactcaatttcacctgcag

SEQ ID NO: 6 - DNA, 57 bp, Baculoviridae
  RHDV/His-R
gcatttcgaatcaatggtggtgatgatggtgacctccgacataagaaaagccattag